European Patent Application EP 4 620 979 A1, published September 24, 2025. Title: 抗体及び抗体を生産する方法. Applicant: Cognano, Inc. The sequence listing filed with the application follows.

SEQUENCE LISTING (75 sequences)

SEQ ID NO: 1 - protein, 113 aa, Vicugna pacos
MAQVQLQESGGGLVQPGGSLRLSCAASGDIFSIYAMGWYRQAPGKQRELVAIVTGLGGTNYADFVKGRFTISRDNAKNTVYLQMNNLIPEDTAVYYCYVRGYWGQGTQVTVSS

SEQ ID NO: 2 - protein, 127 aa, Vicugna pacos
MAQVQLQESGGGSVQPGGSLGLSCAASGSIIRISTMGWYRQIPGQQRELVGDISSGGTTNYADSVKGRFTISRDNAKNTVYLQMNSLKPEDTATYYCYADRITYQRDFLLYAGTGYWGQGTQVTVSS

SEQ ID NO: 3 - protein, 115 aa, Vicugna pacos
MAQVQLQESGGGLVQPGGSLRLSCAASGNIVRFYVMGWYRQAPGKQRELVAQITTGGSALYADSVKGRFTISRDNAKNTVYLQMNSLKPEDTAVYYCNQLPGNSWGQGTQVTVSS

SEQ ID NO: 4 - protein, 124 aa, Vicugna pacos
MAQVQLQESGGGLVQPGGSLRLSCAASGIIFSTYPFSMHTMAWYRQAPGKQRDLVASITVGGSTAYADSVKGRFTISRNNAKKTVELQMNNLGPEDTAAYLCNAKRIGTNEAYWGQGTQVTVSS

SEQ ID NO: 5 - protein, 125 aa, Vicugna pacos
MAQVQLQESGGGLVQPGGSLRLSCAASGINFSRYAMGWYRQAPGEQRELVASITAGGTSKLADPVKGRFTISRDNAKNTVYLQMNSLKPEDTAVYYCNYALGDISAVRPTIFHNWAQGTQVTVSS

SEQ ID NO: 6 - protein, 122 aa, Vicugna pacos
MAQVQLQESGGGLVQPGESLLLSCAVTGIPFSIYTMDWYRQAPGKQRELVAAITSSHRLYYIDSVKGRFTISRDNAKNTVYLQMNSLKPEDTAVYYCSTYTTSAGGSGGRSWGQGTQVTVSS

SEQ ID NO: 7 - protein, 125 aa, Vicugna pacos
MAQVQLQESGGGLVQPGGSLRLSCAASGFTFSSATMSWVRQAPGKGLEWVSGIDSGGRITTYADAVKGRFTIFRDNAKNTLYLQMNSLKPEDTARYYCARGYYYAAESLAKLSFRGQGTQVTVSS

SEQ ID NO: 8 - protein, 122 aa, Vicugna pacos
MAQVQLQESGGGLVQPGGSLRLSCAASGSIFSIYNMRWYRQAPGQQRELVAGITSSGTTVYADSVKGRFTISRDNAKNTVALQMNSLKPEDTAVYYCYAGRRGDNGSMYGYWGQGTQVTVSS

SEQ ID NO: 9 - protein, 117 aa, Vicugna pacos
MAQVQLQESGGGLVQPGGSLRLSCAASGNINSFLSMGWYRQAPGKERELVARFTATGSKNYAEFVKGRFTISRDTAGNTVSLQMNTLKAEDTAVYYCNGIDRRGVYWGQGTQVTVSS

SEQ ID NO: 10 - protein, 116 aa, Vicugna pacos
MAQVQLQESGGGVVEPGGSLTISCTVSGFSLTTYGMTWLRQAPGKGPEWLLSIARGTGTPFYADSVEGRFTASVDSAGNTIYLQMNDLKPEDTALYYCSTASGNYRSPGTQVTVSS

SEQ ID NO: 11 - protein, 119 aa, Vicugna pacos
MAQVQLQESGGGLVQPGGSLRLSCTGSPTIFRGIWMSWVRRAPGKGPEWISSHSPSTPATNYADSVRGRFTISRVNAIGTLYLEMNNLRPEDTARYYCATGGRKDYNIRGQGTQVTVSS

SEQ ID NO: 12 - protein, 116 aa, Vicugna pacos
MAQVQLQESGGGLVQPGGSLKLSCAVSGFALKDYNMAWYRAAAGKNRELVARQSGSGESTTYVPSVKGRFTMTRDNSKNMLYLQMNSLRFDDAAVYYCVRSFDGTSGQGTQVTVSS

SEQ ID NO: 13 - protein, 122 aa, Vicugna pacos
MAQVQLQESGGGSVQPGGSLRLSCAASGFTFGNYAMRWVRQAPGKGPEWVSYVNEAGDSTWYADSVKGRFTITRDNAKNTLYLQMNSLKPEDTALYYCARKPPGGDYAIDYWGKGTQVTVSS

SEQ ID NO: 14 - protein, 122 aa, Vicugna pacos
MAQVQLQESGGGLVQPGGSLRLSCAASGFTFSSYAMSWYRQAPGKERELVATITSAGGRSSYADSVKGRFTISRDNAKNTVYLQMNSLKPEDTAVYYCNAELGPRRHGMDYWGKGTQVTVSS

SEQ ID NO: 15 - protein, 118 aa, Vicugna pacos
MAQVQLQESGGGVVQPGGSLTLSCVASGLALSFSRYIVGWYRQAPGKQRDLVATISSDGDIKYGDSVKGRFNVSRDNVKRTVTLQMNSLKSEDTAVYYCYVRRLATSWGQGTQVTVSS

SEQ ID NO: 16 - protein, 125 aa, Vicugna pacos
MAQVQLQESGGGLVQPGGSLRLSCAASVNLDRYAIGWVRQAPGKEREGVSCVTSGDPETFYEDSVKGRFTISRDNAKNTVFLQMNSLEPEDTAVYYCAAHGGWGLCPRSVSDYDYWGQGTQVTSS

SEQ ID NO: 17 - protein, 114 aa, Vicugna pacos
MAQVQLQESGGGLVQPGGSLRLSCAASGFTFSKYWMTWFRQAPGRGLEWVSDINGGGGTTRYADSVKGRFTISRDNAKNTLYLQMNSLKPEDTAVYYCVNGPSGGQGTQVTVSS

SEQ ID NO: 18 - protein, 5 aa, Vicugna pacos
FSIYA

SEQ ID NO: 19 - protein, 9 aa, Vicugna pacos
IVTGLGGTN

SEQ ID NO: 20 - protein, 5 aa, Vicugna pacos
YVRGY

SEQ ID NO: 21 - protein, 5 aa, Vicugna pacos
IRIST

SEQ ID NO: 22 - protein, 9 aa, Vicugna pacos
DISSGGTTN

SEQ ID NO: 23 - protein, 19 aa, Vicugna pacos
YADRITYQRDFLLYAGTGY

SEQ ID NO: 24 - protein, 5 aa, Vicugna pacos
VRFYV

SEQ ID NO: 25 - protein, 9 aa, Vicugna pacos
QITTGGSAL

SEQ ID NO: 26 - protein, 7 aa, Vicugna pacos
NQLPGNS

SEQ ID NO: 27 - protein, 5 aa, Vicugna pacos
FSTYP

SEQ ID NO: 28 - protein, 14 aa, Vicugna pacos
RDLVASITVGGSTA

SEQ ID NO: 29 - protein, 11 aa, Vicugna pacos
NAKRIGTNEAY

SEQ ID NO: 30 - protein, 5 aa, Vicugna pacos
FSRYA

SEQ ID NO: 31 - protein, 9 aa, Vicugna pacos
SITAGGTSK

SEQ ID NO: 32 - protein, 17 aa, Vicugna pacos
NYALGDISAVRPTIFHN

SEQ ID NO: 33 - protein, 5 aa, Vicugna pacos
FSIYT

SEQ ID NO: 34 - protein, 9 aa, Vicugna pacos
AITSSHRLY

SEQ ID NO: 35 - protein, 14 aa, Vicugna pacos
STYTTSAGGSGGRS

SEQ ID NO: 36 - protein, 5 aa, Vicugna pacos
FSSAT

SEQ ID NO: 37 - protein, 10 aa, Vicugna pacos
GIDSGGRITT

SEQ ID NO: 38 - protein, 16 aa, Vicugna pacos
ARGYYYAAESLAKLSF

SEQ ID NO: 39 - protein, 5 aa, Vicugna pacos
FSIYN

SEQ ID NO: 40 - protein, 9 aa, Vicugna pacos
GITSSGTTV

SEQ ID NO: 41 - protein, 14 aa, Vicugna pacos
YAGRRGDNGSMYGY

SEQ ID NO: 42 - protein, 5 aa, Vicugna pacos
NSFLS

SEQ ID NO: 43 - protein, 9 aa, Vicugna pacos
RFTATGSKN

SEQ ID NO: 44 - protein, 9 aa, Vicugna pacos
NGIDRRGVY

SEQ ID NO: 45 - protein, 5 aa, Vicugna pacos
LTTYG

SEQ ID NO: 46 - protein, 10 aa, Vicugna pacos
SIARGTGTPF

SEQ ID NO: 47 - protein, 7 aa, Vicugna pacos
STASGNY

SEQ ID NO: 48 - protein, 5 aa, Vicugna pacos
FRGIW

SEQ ID NO: 49 - protein, 10 aa, Vicugna pacos
SHSPSTPATN

SEQ ID NO: 50 - protein, 10 aa, Vicugna pacos
ATGGRKDYNI

SEQ ID NO: 51 - protein, 5 aa, Vicugna pacos
LKDYN

SEQ ID NO: 52 - protein, 10 aa, Vicugna pacos
RQSGSGESTT

SEQ ID NO: 53 - protein, 7 aa, Vicugna pacos
VRSFDGT

SEQ ID NO: 54 - protein, 5 aa, Vicugna pacos
FGNYA

SEQ ID NO: 55 - protein, 10 aa, Vicugna pacos
YVNEAGDSTW

SEQ ID NO: 56 - protein, 13 aa, Vicugna pacos
ARKPPGGDYAIDY

SEQ ID NO: 57 - protein, 5 aa, Vicugna pacos
FSSYA

SEQ ID NO: 58 - protein, 10 aa, Vicugna pacos
TITSAGGRSS

SEQ ID NO: 59 - protein, 13 aa, Vicugna pacos
NAELGPRRHGMDY

SEQ ID NO: 60 - protein, 7 aa, Vicugna pacos
LSFSRYI

SEQ ID NO: 61 - protein, 9 aa, Vicugna pacos
TISSDGDIK

SEQ ID NO: 62 - protein, 8 aa, Vicugna pacos
YVRRLATS

SEQ ID NO: 63 - protein, 4 aa, Vicugna pacos
DRYA

SEQ ID NO: 64 - protein, 10 aa, Vicugna pacos
CVTSGDPETF

SEQ ID NO: 65 - protein, 18 aa, Vicugna pacos
AAHGGWGLCPRSVSDYDY

SEQ ID NO: 66 - protein, 5 aa, Vicugna pacos
FSKYW

SEQ ID NO: 67 - protein, 10 aa, Vicugna pacos
DINGGGGTTR

SEQ ID NO: 68 - protein, 5 aa, Vicugna pacos
VNGPS

SEQ ID NO: 69 - DNA, 23 bp, synthetic construct
  misc_feature 1..23: note = Primer Sequence
  source 1..23: mol_type = other DNA
gtcctggctgctcttctacaagg

SEQ ID NO: 70 - DNA, 23 bp, synthetic construct
  misc_feature 1..23: note = Primer Sequence
  source 1..23: mol_type = other DNA
ggtacgtgctgttgaactgttcc

SEQ ID NO: 71 - DNA, 21 bp, synthetic construct
  misc_feature 1..21: note = Primer Sequence
  source 1..21: mol_type = other DNA
gaaatacctattgcctacggc

SEQ ID NO: 72 - DNA, 21 bp, synthetic construct
  misc_feature 1..21: note = Primer Sequence
  source 1..21: mol_type = other DNA
ggaaccgtagtccggaacgtc

SEQ ID NO: 73 - DNA, 33 bp, synthetic construct
  misc_feature 1..33: note = Primer Sequence
  source 1..33: mol_type = other DNA
tcgtcggcagcgtcagatgtgtataagagacag

SEQ ID NO: 74 - DNA, 34 bp, synthetic construct
  misc_feature 1..34: note = Primer Sequence
  source 1..34: mol_type = other DNA
gtctcgtgggctcggagatgtgtataagagacag

SEQ ID NO: 75 - protein, 20 aa, synthetic construct
GGGGSGGGGSGGGGSGGGGS